European Patent Application EP 4 772 525 A1, published July 8, 2026. Title: Novel Peptide Having Activity of Improving Skin Condition and Uses Thereof. Applicant: CAREGEN CO., LTD. Application KR. The sequence listing filed with the application follows.

SEQUENCE LISTING (9 sequences)

SEQ ID NO: 1 - protein, 8 aa, synthetic construct
GWGDPIRL

SEQ ID NO: 2 - DNA, 20 bp, synthetic construct
  source 1..20: mol_type = other DNA
caccctcaagagcctgagtc

SEQ ID NO: 3 - DNA, 20 bp, synthetic construct
  source 1..20: mol_type = other DNA
agacggctgagtagggaaca

SEQ ID NO: 4 - DNA, 20 bp, synthetic construct
  source 1..20: mol_type = other DNA
ccaggaaccgagtacaccat

SEQ ID NO: 5 - DNA, 20 bp, synthetic construct
  source 1..20: mol_type = other DNA
atacccaggttgggtgatga

SEQ ID NO: 6 - DNA, 20 bp, synthetic construct
  source 1..20: mol_type = other DNA
gcaagacctggctttggact

SEQ ID NO: 7 - DNA, 21 bp, synthetic construct
  source 1..21: mol_type = other DNA
gggagtttctggttagggctg

SEQ ID NO: 8 - DNA, 20 bp, synthetic construct
  source 1..20: mol_type = other DNA
ggagccaaaagggtcatcat

SEQ ID NO: 9 - DNA, 20 bp, synthetic construct
  source 1..20: mol_type = other DNA
gtgatggcatggactgtggt